European Patent Application EP 4 527 999 A1, published March 26, 2025. Title: 嵩高混紡糸及びその製造方法. Applicant: スパイバー株式会社. Application JP. The sequence listing filed with the application follows.

SEQUENCE LISTING (8 sequences)

SEQ ID NO: 1 - protein, 2375 aa, synthetic construct
MHHHHHHSSGSSGPGQQGPYGPGASAAAAAGQNGPGSGQQGPGQSGQYGPGQQGPGQQGPGSSAAAAAGPGQYGPGQQGPSASAAAAAGPGSGQQGPGASGQYGPGQQGPGQQGPGSSAAAAAGQYGSGPGQQGPYGSAAAAAGPGSGQYGQGPYGPGASGPGQYGPGQQGPSASAAAAAGSGQQGPGQYGPYASAAAAAGQYGSGPGQQGPYGPGQSGSGQQGPGQQGPYASAAAAAGPGQQGPYGPGSSAAAAAGQYGYGPGQQGPYGPGASGQNGPGSGQYGPGQQGPGQSAAAAAGPGQQGPYGPGASAAAAAGQYGPGQQGPGQYGPGSSGPGQQGPYGPGSSAAAAAGQYGPGQQGPYGPGQSAAAAAGQYQQGPGQQGPYGPGASGPGQQGPYGPGASAAAAAGPGQYGPGQQGPSASAAAAAGQYGSGPGQYGPYGPGQSGPGSGQQGQGPYGPGASAAAAAGQYGPGQQGPYGPGQSAAAAAGPGSGQYGPGASGQNGPGSGQYGPGQQGPGQSAAAAAGQYQQGPGQQGPYGPGASAAAAAGQYGSGPGQQGPYGPGQSGSGQQGPGQQGPYASAAAAAGPGSGQQGPGASGQQGPYGPGASAAAAAGQNGPGSGQQGPGQSGQYGPGQQGPGQQGPGSSAAAAAGPGQYGPGQQGPSASAAAAAGPGSGQQGPGASGQYGPGQQGPGQQGPGSSAAAAAGQYGSGPGQQGPYGSAAAAAGPGSGQYGQGPYGPGASGPGQYGPGQQGPSASAAAAAGSGQQGPGQYGPYASAAAAAGQYGSGPGQQGPYGPGQSGSGQQGPGQQGPYASAAAAAGPGQQGPYGPGSSAAAAAGQYGYGPGQQGPYGPGASGQNGPGSGQYGPGQQGPGQSAAAAAGPGQQGPYGPGASAAAAAGQYGPGQQGPGQYGPGSSGPGQQGPYGPGSSAAAAAGQYGPGQQGPYGPGQSAAAAAGQYQQGPGQQGPYGPGASGPGQQGPYGPGASAAAAAGPGQYGPGQQGPSASAAAAAGQYGSGPGQYGPYGPGQSGPGSGQQGQGPYGPGASAAAAAGQYGPGQQGPYGPGQSAAAAAGPGSGQYGPGASGQNGPGSGQYGPGQQGPGQSAAAAAGQYQQGPGQQGPYGPGASAAAAAGQYGSGPGQQGPYGPGQSGSGQQGPGQQGPYASAAAAAGPGSGQQGPGASGQQGPYGPGASAAAAAGQNGPGSGQQGPGQSGQYGPGQQGPGQQGPGSSAAAAAGPGQYGPGQQGPSASAAAAAGPGSGQQGPGASGQYGPGQQGPGQQGPGSSAAAAAGQYGSGPGQQGPYGSAAAAAGPGSGQYGQGPYGPGASGPGQYGPGQQGPSASAAAAAGSGQQGPGQYGPYASAAAAAGQYGSGPGQQGPYGPGQSGSGQQGPGQQGPYASAAAAAGPGQQGPYGPGSSAAAAAGQYGYGPGQQGPYGPGASGQNGPGSGQYGPGQQGPGQSAAAAAGPGQQGPYGPGASAAAAAGQYGPGQQGPGQYGPGSSGPGQQGPYGPGSSAAAAAGQYGPGQQGPYGPGQSAAAAAGQYQQGPGQQGPYGPGASGPGQQGPYGPGASAAAAAGPGQYGPGQQGPSASAAAAAGQYGSGPGQYGPYGPGQSGPGSGQQGQGPYGPGASAAAAAGQYGPGQQGPYGPGQSAAAAAGPGSGQYGPGASGQNGPGSGQYGPGQQGPGQSAAAAAGQYQQGPGQQGPYGPGASAAAAAGQYGSGPGQQGPYGPGQSGSGQQGPGQQGPYASAAAAAGPGSGQQGPGASGQQGPYGPGASAAAAAGQNGPGSGQQGPGQSGQYGPGQQGPGQQGPGSSAAAAAGPGQYGPGQQGPSASAAAAAGPGSGQQGPGASGQYGPGQQGPGQQGPGSSAAAAAGQYGSGPGQQGPYGSAAAAAGPGSGQYGQGPYGPGASGPGQYGPGQQGPSASAAAAAGSGQQGPGQYGPYASAAAAAGQYGSGPGQQGPYGPGQSGSGQQGPGQQGPYASAAAAAGPGQQGPYGPGSSAAAAAGQYGYGPGQQGPYGPGASGQNGPGSGQYGPGQQGPGQSAAAAAGPGQQGPYGPGASAAAAAGQYGPGQQGPGQYGPGSSGPGQQGPYGPGSSAAAAAGQYGPGQQGPYGPGQSAAAAAGQYQQGPGQQGPYGPGASGPGQQGPYGPGASAAAAAGPGQYGPGQQGPSASAAAAAGQYGSGPGQYGPYGPGQSGPGSGQQGQGPYGPGASAAAAAGQYGPGQQGPYGPGQSAAAAAGPGSGQYGPGASGQNGPGSGQYGPGQQGPGQSAAAAAGQYQQGPGQQGPYGPGASAAAAAGQYGSGPGQQGPYGPGQSGSGQQGPGQQGPYASAAAAAGPGSGQQGSSVDKLAAALEHHHHHH

SEQ ID NO: 2 - protein, 1190 aa, synthetic construct
MHHHHHHSSGSSGPGVFGPYGPGASAAAAAGINGPGSGVFGPGISGIYGPGVFGPGVFGPGSSAAAAAGPGIYGPGVFGPSASAAAAAGPGSGVFGPGASGIYGPGVFGPGVFGPGSSAAAAAGIYGSGPGVFGPYGSAAAAAGPGSGIYGIGPYGPGASGPGIYGPGVFGPSASAAAAAGSGVFGPGIYGPYASAAAAAGIYGSGPGVFGPYGPGISGSGVFGPGVFGPYASAAAAAGPGVFGPYGPGSSAAAAAGIYGYGPGVFGPYGPGASGINGPGSGIYGPGVFGPGISAAAAAGPGVFGPYGPGASAAAAAGIYGPGVFGPGIYGPGSSGPGVFGPYGPGSSAAAAAGIYGPGVFGPYGPGISAAAAAGIYVFGPGVFGPYGPGASGPGVFGPYGPGASAAAAAGPGIYGPGVFGPSASAAAAAGIYGSGPGIYGPYGPGISGPGSGVFGIGPYGPGASAAAAAGIYGPGVFGPYGPGISAAAAAGPGSGIYGPGASGINGPGSGIYGPGVFGPGISAAAAAGIYVFGPGVFGPYGPGASAAAAAGIYGSGPGVFGPYGPGISGSGVFGPGVFGPYASAAAAAGPGSGVFGPGASGPGVFGPYGPGASAAAAAGINGPGSGVFGPGISGIYGPGVFGPGVFGPGSSAAAAAGPGIYGPGVFGPSASAAAAAGPGSGVFGPGASGIYGPGVFGPGVFGPGSSAAAAAGIYGSGPGVFGPYGSAAAAAGPGSGIYGIGPYGPGASGPGIYGPGVFGPSASAAAAAGSGVFGPGIYGPYASAAAAAGIYGSGPGVFGPYGPGISGSGVFGPGVFGPYASAAAAAGPGVFGPYGPGSSAAAAAGIYGYGPGVFGPYGPGASGINGPGSGIYGPGVFGPGISAAAAAGPGVFGPYGPGASAAAAAGIYGPGVFGPGIYGPGSSGPGVFGPYGPGSSAAAAAGIYGPGVFGPYGPGISAAAAAGIYVFGPGVFGPYGPGASGPGVFGPYGPGASAAAAAGPGIYGPGVFGPSASAAAAAGIYGSGPGIYGPYGPGISGPGSGVFGIGPYGPGASAAAAAGIYGPGVFGPYGPGISAAAAAGPGSGIYGPGASGINGPGSGIYGPGVFGPGISAAAAAGIYVFGPGVFGPYGPGASAAAAAGIYGSGPGVFGPYGPGISGSGVFGPGVFGPYASAAAAAGPGSGVFGPGAS

SEQ ID NO: 3 - protein, 601 aa, synthetic construct
MHHHHHHSSGSSGPGVFGPYGPGASAAAAAGINGPGSGVFGPGISGIYGPGVFGPGVFGPGSSAAAAAGPGIYGPGVFGPSASAAAAAGPGSGVFGPGASGIYGPGVFGPGVFGPGSSAAAAAGIYGSGPGVFGPYGSAAAAAGPGSGIYGIGPYGPGASGPGIYGPGVFGPSASAAAAAGSGVFGPGIYGPYASAAAAAGIYGSGPGVFGPYGPGISGSGVFGPGVFGPYASAAAAAGPGVFGPYGPGSSAAAAAGIYGYGPGVFGPYGPGASGINGPGSGIYGPGVFGPGISAAAAAGPGVFGPYGPGASAAAAAGIYGPGVFGPGIYGPGSSGPGVFGPYGPGSSAAAAAGIYGPGVFGPYGPGISAAAAAGIYVFGPGVFGPYGPGASGPGVFGPYGPGASAAAAAGPGIYGPGVFGPSASAAAAAGIYGSGPGIYGPYGPGISGPGSGVFGIGPYGPGASAAAAAGIYGPGVFGPYGPGISAAAAAGPGSGIYGPGASGINGPGSGIYGPGVFGPGISAAAAAGIYVFGPGVFGPYGPGASAAAAAGIYGSGPGVFGPYGPGISGSGVFGPGVFGPYASAAAAAGPGSGVFGPGAS

SEQ ID NO: 4 - protein, 608 aa, synthetic construct
MHHHHHHSSGSSGPGGQGPYGPGASAAAAAGGNGPGSGQQGPGGSAAAAAGGYGPGGQGPGQQGPGSSAAAAAGPGGYGPGGQGPSASAAAAAGPGSGQQGPGASAAAAAGGYGPGGQGPGQQGPGSSAAAAAGGYGSGPGQQGPYGSAAAAAGPGSGGYGQGPYGPGASAAAAAGPGGYGPGGQGPSASAAAAAGSGQQGPGGYGPYASAAAAAGGYGSGPGQQGPYGPGGSAAAAAGSGQQGPGQQGPYASAAAAAGPGGQGPYGPGSSAAAAAGGYGYGPGGQGPYGPGASAAAAAGGNGPGSGGYGPGQQGPGGSAAAAAGPGGQGPYGPGASAAAAAGGYGPGGQGPGGYGPGSSAAAAAGPGGQGPYGPGSSAAAAAGGYGPGQQGPYGPGGSAAAAAGGYQQGPGGQGPYGPGASAAAAAGPGGQGPYGPGASAAAAAGPGGYGPGGQGPSASAAAAAGGYGSGPGGYGPYGPGGSAAAAAGPGSGQQGQGPYGPGASAAAAAGGYGPGQQGPYGPGGSAAAAAGPGSGGYGPGASAAAAAGGNGPGSGGYGPGQQGPGGSAAAAAGGYQQGPGGQGPYGPGASAAAAAGPGSGQQGPGAS

SEQ ID NO: 5 - protein, 603 aa, synthetic construct
MHHHHHHSSGSSCGPGVFGPYGPGASAAAAAGINGPGSGVFGPGISGIYGPGVFGPGVFGPGSSAAAAAGPGIYGPGVFGPSASAAAAAGPGSGVFGPGASGIYGPGVFGPGVFGPGSSAAAAAGIYGSGPGVFGPYGSAAAAAGPGSGIYGIGPYGPGASGPGIYGPGVFGPSASAAAAAGSGVFGPGIYGPYASAAAAAGIYGSGPGVFGPYGPGISGSGVFGPGVFGPYASAAAAAGPGVFGPYGPGSSAAAAAGIYGYGPGVFGPYGPGASGINGPGSGIYGPGVFGPGISAAAAAGPGVFGPYGPGASAAAAAGIYGPGVFGPGIYGPGSSGPGVFGPYGPGSSAAAAAGIYGPGVFGPYGPGISAAAAAGIYVFGPGVFGPYGPGASGPGVFGPYGPGASAAAAAGPGIYGPGVFGPSASAAAAAGIYGSGPGIYGPYGPGISGPGSGVFGIGPYGPGASAAAAAGIYGPGVFGPYGPGISAAAAAGPGSGIYGPGASGINGPGSGIYGPGVFGPGISAAAAAGIYVFGPGVFGPYGPGASAAAAAGIYGSGPGVFGPYGPGISGSGVFGPGVFGPYASAAAAAGPGCSGVFGPGAS

SEQ ID NO: 6 - protein, 605 aa, synthetic construct
MHHHHHHSSGSSCGPGVFGPYGPGASAAAAAGINGPGSGVFGPGISCGIYGPGVFGPGVFGPGSSAAAAAGPGIYGPGVFGPSASAAAAAGPGSGVFGPGASGIYGPGVFGPGVFGPGSSAAAAAGIYGSGPGVFGPYGSAAAAAGPGSGIYGIGPYGPGASGPGIYGPGVFGPSASAAAAAGSGVFGPGIYGPYASAAAAAGIYGSGPGVFGPYGPGISGSGVFGPGVFGPYASAAAAAGPGVFGPYGPGSSAAAAAGIYGYGPGVFGPYGPGASGINGPGSGIYGPGVFGPGISAAAAAGPGVFGPYGPGASAAAAAGIYGPGVFGPGIYGPGSSGPGVFGPYGPGSSAAAAAGIYGPGVFGPYGPGISAAAAAGIYVFGPGVFGPYGPGASGPGVFGPYGPGASAAAAAGPGIYGPGVFGPSASAAAAAGIYGSGPGIYGPYGPGISGPGSGVFGIGPYGPGASAAAAAGIYGPGVFGPYGPGISAAAAAGPGSGIYGPGASGINGPGSGIYGPGVFGPGISAAAAAGIYVFGPGVFGPYGPGASAAAAAGIYGSGPGVFGPYGPGISGCSGVFGPGVFGPYASAAAAAGPGCSGVFGPGAS

SEQ ID NO: 7 - protein, 1188 aa, synthetic construct
MHHHHHHSSGSSGPGQQGPYGPGASAAAAAGQNGPGSGQQGPGQSGQYGPGQQGPGQQGPGSSAAAAAGPGQYGPGQQGPSASAAAAAGPGSGQQGPGASGQYGPGQQGPGQQGPGSSAAAAAGQYGSGPGQQGPYGSAAAAAGPGSGQYGQGPYGPGASGPGQYGPGQQGPSASAAAAAGSGQQGPGQYGPYASAAAAAGQYGSGPGQQGPYGPGQSGSGQQGPGQQGPYASAAAAAGPGQQGPYGPGSSAAAAAGQYGYGPGQQGPYGPGASGQNGPGSGQYGPGQQGPGQSAAAAAGPGQQGPYGPGASAAAAAGQYGPGQQGPGQYGPGSSGPGQQGPYGPGSSAAAAAGQYGPGQQGPYGPGQSAAAAAGQYQQGPGQQGPYGPGASGPGQQGPYGPGASAAAAAGPGQYGPGQQGPSASAAAAAGQYGSGPGQYGPYGPGQSGPGSGQQGQGPYGPGASAAAAAGQYGPGQQGPYGPGQSAAAAAGPGSGQYGPGASGQNGPGSGQYGPGQQGPGQSAAAAAGQYQQGPGQQGPYGPGASAAAAAGQYGSGPGQQGPYGPGQSGSGQQGPGQQGPYASAAAAAGPGSGQQGPGASGQQGPYGPGASAAAAAGQNGPGSGQQGPGQSGQYGPGQQGPGQQGPGSSAAAAAGPGQYGPGQQGPSASAAAAAGPGSGQQGPGASGQYGPGQQGPGQQGPGSSAAAAAGQYGSGPGQQGPYGSAAAAAGPGSGQYGQGPYGPGASGPGQYGPGQQGPSASAAAAAGSGQQGPGQYGPYASAAAAAGQYGSGPGQQGPYGPGQSGSGQQGPGQQGPYASAAAAAGPGQQGPYGPGSSAAAAAGQYGYGPGQQGPYGPGASGQNGPGSGQYGPGQQGPGQSAAAAAGPGQQGPYGPGASAAAAAGQYGPGQQGPGQYGPGSSGPGQQGPYGPGSSAAAAAGQYGPGQQGPYGPGQSAAAAAGQYQQGPGQQGPYGPGASGPGQQGPYGPGASAAAAAGPGQYGPGQQGPSASAAAAAGQYGSGPGQYGPYGPGQSGPGSGQQGQGPYGPGASAAAAAGQYGPGQQGPYGPGQSAAAAAGPGSGQYGPGASGQNGPGSGQYGPGQQGPGQSAAAAAGQYQQGPGQQGPYGPGASAAAAAGQYGSGPGQQGPYGPGQSGSGQQGPGQQGPYASAAAAAGPGSGQQGPGAS

SEQ ID NO: 8 - protein, 24 aa, synthetic construct
MHHHHHHHHHHSSGSSLEVLFQGP